European Patent Specification EP 3 122 365 B1, published May 3, 2023. Title: TRANSTHYRETIN ALLELE SELECTIVE UNA OLIGOMERS FOR GENE SILENCING. Applicant: ARCTURUS THERAPEUTICS, INC. The sequence listing filed with the application follows.

SEQUENCE LISTING (72 sequences)

SEQ ID NO: 1 - RNA, 22 nt, Artificial Sequence
  Description of Artificial Sequence: Synthetic oligonucleotide
  modified_base (1)..(1): UNA monomer
  modified_base (2)..(20): a, c, u, g, unknown or other
  modified_base (21)..(22): UNA monomer
nnnnnnnnnnnnnnnnnnnnnn

SEQ ID NO: 2 - RNA, 21 nt, Artificial Sequence
  Description of Artificial Sequence: Synthetic oligonucleotide
  modified_base (1)..(1): a, c, u, g, unknown or other
  modified_base (2)..(8): UNA monomer
  modified_base (9)..(19): a, c, u, g, unknown or other
  modified_base (20)..(21): UNA monomer
nnnnnnnnnnnnnnnnnnnnn

SEQ ID NO: 3 - RNA, 21 nt, Artificial Sequence
  Description of Artificial Sequence: Synthetic P15U6 oligonucleotide
  modified_base (1)..(1): Non-nucleotide monomer
  modified_base (20)..(20): Non-nucleotide monomer
ggccaugcauguguucagauu

SEQ ID NO: 4 - RNA, 21 nt, Artificial Sequence
  Description of Artificial Sequence: Synthetic P15U6 oligonucleotide
  modified_base (6)..(6): Non-nucleotide monomer
  modified_base (20)..(20): Non-nucleotide monomer
ucugaacacaugcauggccuu

SEQ ID NO: 5 - RNA, 21 nt, Artificial Sequence
  Description of Artificial Sequence: Synthetic P15U7 oligonucleotide
  modified_base (1)..(1): Non-nucleotide monomer
  modified_base (20)..(20): Non-nucleotide monomer
ggccaugcauguguucagauu

SEQ ID NO: 6 - RNA, 21 nt, Artificial Sequence
  Description of Artificial Sequence: Synthetic P15U7 oligonucleotide
  modified_base (7)..(7): Non-nucleotide monomer
  modified_base (20)..(20): Non-nucleotide monomer
ucugaacacaugcauggccuu

SEQ ID NO: 7 - RNA, 21 nt, Artificial Sequence
  Description of Artificial Sequence: Synthetic P15U14 oligonucleotide
  modified_base (1)..(1): Non-nucleotide monomer
  modified_base (20)..(20): Non-nucleotide monomer
ggccaugcauguguucagauu

SEQ ID NO: 8 - RNA, 21 nt, Artificial Sequence
  Description of Artificial Sequence: Synthetic P15U14 oligonucleotide
  modified_base (14)..(14): Non-nucleotide monomer
  modified_base (20)..(20): Non-nucleotide monomer
ucugaacacaugcauggccuu

SEQ ID NO: 9 - RNA, 21 nt, Artificial Sequence
  Description of Artificial Sequence: Synthetic P15U15 oligonucleotide
  modified_base (1)..(1): Non-nucleotide monomer
  modified_base (20)..(20): Non-nucleotide monomer
ggccaugcauguguucagauu

SEQ ID NO: 10 - RNA, 21 nt, Artificial Sequence
  Description of Artificial Sequence: Synthetic P15U15 oligonucleotide
  modified_base (15)..(15): Non-nucleotide monomer
  modified_base (20)..(20): Non-nucleotide monomer
ucugaacacaugcauggccuu

SEQ ID NO: 11 - RNA, 21 nt, Artificial Sequence
  Description of Artificial Sequence: Synthetic P15U16 oligonucleotide
  modified_base (1)..(1): Non-nucleotide monomer
  modified_base (20)..(20): Non-nucleotide monomer
ggccaugcauguguucagauu

SEQ ID NO: 12 - RNA, 21 nt, Artificial Sequence
  Description of Artificial Sequence: Synthetic P15U16 oligonucleotide
  modified_base (16)..(16): Non-nucleotide monomer
  modified_base (20)..(20): Non-nucleotide monomer
ucugaacacaugcauggccuu

SEQ ID NO: 13 - RNA, 21 nt, Artificial Sequence
  Description of Artificial Sequence: Synthetic P16U6 oligonucleotide
  modified_base (1)..(1): Non-nucleotide monomer
  modified_base (20)..(20): Non-nucleotide monomer
gccaugcauguguucagaauu

SEQ ID NO: 14 - RNA, 21 nt, Artificial Sequence
  Description of Artificial Sequence: Synthetic P16U6 oligonucleotide
  modified_base (6)..(6): Non-nucleotide monomer
  modified_base (20)..(20): Non-nucleotide monomer
uucugaacacaugcauggcuu

SEQ ID NO: 15 - RNA, 21 nt, Artificial Sequence
  Description of Artificial Sequence: Synthetic P16U7 oligonucleotide
  modified_base (1)..(1): Non-nucleotide monomer
  modified_base (20)..(20): Non-nucleotide monomer
gccaugcauguguucagaauu

SEQ ID NO: 16 - RNA, 21 nt, Artificial Sequence
  Description of Artificial Sequence: Synthetic P16U7 oligonucleotide
  modified_base (7)..(7): Non-nucleotide monomer
  modified_base (20)..(20): Non-nucleotide monomer
uucugaacacaugcauggcuu

SEQ ID NO: 17 - RNA, 21 nt, Artificial Sequence
  Description of Artificial Sequence: Synthetic P16U15 oligonucleotide
  modified_base (1)..(1): Non-nucleotide monomer
  modified_base (20)..(20): Non-nucleotide monomer
gccaugcauguguucagaauu

SEQ ID NO: 18 - RNA, 21 nt, Artificial Sequence
  Description of Artificial Sequence: Synthetic P16U15 oligonucleotide
  modified_base (15)..(15): Non-nucleotide monomer
  modified_base (20)..(20): Non-nucleotide monomer
uucugaacacaugcauggcuu

SEQ ID NO: 19 - RNA, 21 nt, Artificial Sequence
  Description of Artificial Sequence: Synthetic P16U16 oligonucleotide
  modified_base (1)..(1): Non-nucleotide monomer
  modified_base (20)..(20): Non-nucleotide monomer
gccaugcauguguucagaauu

SEQ ID NO: 20 - RNA, 21 nt, Artificial Sequence
  Description of Artificial Sequence: Synthetic P16U16 oligonucleotide
  modified_base (16)..(16): Non-nucleotide monomer
  modified_base (20)..(20): Non-nucleotide monomer
uucugaacacaugcauggcuu

SEQ ID NO: 21 - RNA, 21 nt, Artificial Sequence
  Description of Artificial Sequence: Synthetic P16U17 oligonucleotide
  modified_base (1)..(1): Non-nucleotide monomer
  modified_base (20)..(20): Non-nucleotide monomer
gccaugcauguguucagaauu

SEQ ID NO: 22 - RNA, 21 nt, Artificial Sequence
  Description of Artificial Sequence: Synthetic P16U17 oligonucleotide
  modified_base (17)..(17): Non-nucleotide monomer
  modified_base (20)..(20): Non-nucleotide monomer
uucugaacacaugcauggcuu

SEQ ID NO: 23 - RNA, 41 nt, Artificial Sequence
  Description of Artificial Sequence: Synthetic V30M TTR oligonucleotide
guccugccaucaauguggccaugcauguguucagaaaggcu

SEQ ID NO: 24 - RNA, 41 nt, Unknown
  Description of Unknown: wt TTR oligonucleotide
guccugccaucaauguggccgugcauguguucagaaaggcu

SEQ ID NO: 25 - DNA, 21 bp, Artificial Sequence
  Description of Artificial Sequence: Synthetic V30V-P2 oligonucleotide
  Description of Combined DNA/RNA Molecule: Synthetic V30V-P2 oligonucleotide
acggccacauugauggcagtt

SEQ ID NO: 26 - DNA, 21 bp, Artificial Sequence
  Description of Artificial Sequence: Synthetic V30V-P3 oligonucleotide
  Description of Combined DNA/RNA Molecule: Synthetic V30V-P3 oligonucleotide
cacggccacauugauggcatt

SEQ ID NO: 27 - DNA, 21 bp, Artificial Sequence
  Description of Artificial Sequence: Synthetic V30V-P4 oligonucleotide
  Description of Combined DNA/RNA Molecule: Synthetic V30V-P4 oligonucleotide
gcacggccacauugauggctt

SEQ ID NO: 28 - DNA, 21 bp, Artificial Sequence
  Description of Artificial Sequence: Synthetic V30V-P5 oligonucleotide
  Description of Combined DNA/RNA Molecule: Synthetic V30V-P5 oligonucleotide
ugcacggccacauugauggtt

SEQ ID NO: 29 - DNA, 21 bp, Artificial Sequence
  Description of Artificial Sequence: Synthetic V30V-P6 oligonucleotide
  Description of Combined DNA/RNA Molecule: Synthetic V30V-P6 oligonucleotide
augcacggccacauugaugtt

SEQ ID NO: 30 - DNA, 21 bp, Artificial Sequence
  Description of Artificial Sequence: Synthetic V30V-P7 oligonucleotide
  Description of Combined DNA/RNA Molecule: Synthetic V30V-P7 oligonucleotide
caugcacggccacauugautt

SEQ ID NO: 31 - DNA, 21 bp, Artificial Sequence
  Description of Artificial Sequence: Synthetic V30V-P8 oligonucleotide
  Description of Combined DNA/RNA Molecule: Synthetic V30V-P8 oligonucleotide
acaugcacggccacauugatt

SEQ ID NO: 32 - DNA, 21 bp, Artificial Sequence
  Description of Artificial Sequence: Synthetic V30V-P9 oligonucleotide
  Description of Combined DNA/RNA Molecule: Synthetic V30V-P9 oligonucleotide
cacaugcacggccacauugtt

SEQ ID NO: 33 - DNA, 21 bp, Artificial Sequence
  Description of Artificial Sequence: Synthetic V30V-P10 oligonucleotide
  Description of Combined DNA/RNA Molecule: Synthetic V30V-P10 oligonucleotide
acacaugcacggccacauutt

SEQ ID NO: 34 - DNA, 21 bp, Artificial Sequence
  Description of Artificial Sequence: Synthetic V30V-P11 oligonucleotide
  Description of Combined DNA/RNA Molecule: Synthetic V30V-P11 oligonucleotide
aacacaugcacggccacautt

SEQ ID NO: 35 - DNA, 21 bp, Artificial Sequence
  Description of Artificial Sequence: Synthetic V30V-P12 oligonucleotide
  Description of Combined DNA/RNA Molecule: Synthetic V30V-P12 oligonucleotide
gaacacaugcacggccacatt

SEQ ID NO: 36 - DNA, 21 bp, Artificial Sequence
  Description of Artificial Sequence: Synthetic V30V-P13 oligonucleotide
  Description of Combined DNA/RNA Molecule: Synthetic V30V-P13 oligonucleotide
ugaacacaugcacggccactt

SEQ ID NO: 37 - DNA, 21 bp, Artificial Sequence
  Description of Artificial Sequence: Synthetic V30V-P14 oligonucleotide
  Description of Combined DNA/RNA Molecule: Synthetic V30V-P14 oligonucleotide
cugaacacaugcacggccatt

SEQ ID NO: 38 - DNA, 21 bp, Artificial Sequence
  Description of Artificial Sequence: Synthetic V30V-P15 oligonucleotide
  Description of Combined DNA/RNA Molecule: Synthetic V30V-P15 oligonucleotide
ucugaacacaugcacggcctt

SEQ ID NO: 39 - RNA, 41 nt, Artificial Sequence; identical to SEQ ID NO: 23
  Description of Artificial Sequence: Synthetic V30M TTR oligonucleotide

SEQ ID NO: 40 - RNA, 41 nt, Unknown; identical to SEQ ID NO: 24
  Description of Unknown: wt TTR oligonucleotide

SEQ ID NO: 41 - DNA, 21 bp, Artificial Sequence
  Description of Artificial Sequence: Synthetic V30V-P5 oligonucleotide
  Description of Combined DNA/RNA Molecule: Synthetic V30V-P5 oligonucleotide
ugcacggccacauugauggtt

SEQ ID NO: 42 - DNA, 21 bp, Artificial Sequence
  Description of Artificial Sequence: Synthetic V30V-P9 oligonucleotide
  Description of Combined DNA/RNA Molecule: Synthetic V30V-P9 oligonucleotide
cacaugcacggccacauugtt

SEQ ID NO: 43 - DNA, 21 bp, Artificial Sequence
  Description of Artificial Sequence: Synthetic V30V-P14 oligonucleotide
  Description of Combined DNA/RNA Molecule: Synthetic V30V-P14 oligonucleotide
cugaacacaugcacggccatt

SEQ ID NO: 44 - DNA, 21 bp, Artificial Sequence
  Description of Artificial Sequence: Synthetic V30V-P15 oligonucleotide
  Description of Combined DNA/RNA Molecule: Synthetic V30V-P15 oligonucleotide
ucugaacacaugcacggcctt

SEQ ID NO: 45 - DNA, 21 bp, Artificial Sequence
  Description of Artificial Sequence: Synthetic V30M-P5 oligonucleotide
  Description of Combined DNA/RNA Molecule: Synthetic V30M-P5 oligonucleotide
ugcauggccacauugauggtt

SEQ ID NO: 46 - DNA, 21 bp, Artificial Sequence
  Description of Artificial Sequence: Synthetic V30M-P9 oligonucleotide
  Description of Combined DNA/RNA Molecule: Synthetic V30M-P9 oligonucleotide
cacaugcauggccacauugtt

SEQ ID NO: 47 - DNA, 21 bp, Artificial Sequence
  Description of Artificial Sequence: Synthetic V30M-P14 oligonucleotide
  Description of Combined DNA/RNA Molecule: Synthetic V30M-P14 oligonucleotide
cugaacacaugcauggccatt

SEQ ID NO: 48 - DNA, 21 bp, Artificial Sequence
  Description of Artificial Sequence: Synthetic V30M-P15 oligonucleotide
  Description of Combined DNA/RNA Molecule: Synthetic V30M-P15 oligonucleotide
ucugaacacaugcauggcctt

SEQ ID NO: 49 - DNA, 21 bp, Artificial Sequence
  Description of Artificial Sequence: Synthetic siRNA P15 sense oligonucleotide
  Description of Combined DNA/RNA Molecule: Synthetic siRNA P15 sense oligonucleotide
ggccaugcauguguucagatt

SEQ ID NO: 50 - RNA, 21 nt, Artificial Sequence
  Description of Artificial Sequence: Synthetic P15U6 sense oligonucleotide
  modified_base (1)..(1): Non-nucleotide monomer
  modified_base (20)..(20): Non-nucleotide monomer
ggccaugcauguguucagauu

SEQ ID NO: 51 - RNA, 21 nt, Artificial Sequence
  Description of Artificial Sequence: Synthetic P15U7 sense oligonucleotide
  modified_base (1)..(1): Non-nucleotide monomer
  modified_base (20)..(20): Non-nucleotide monomer
ggccaugcauguguucagauu

SEQ ID NO: 52 - RNA, 21 nt, Artificial Sequence
  Description of Artificial Sequence: Synthetic P15U14 sense oligonucleotide
  modified_base (1)..(1): Non-nucleotide monomer
  modified_base (20)..(20): Non-nucleotide monomer
ggccaugcauguguucagauu

SEQ ID NO: 53 - RNA, 21 nt, Artificial Sequence
  Description of Artificial Sequence: Synthetic P15U15 sense oligonucleotide
  modified_base (1)..(1): Non-nucleotide monomer
  modified_base (20)..(20): Non-nucleotide monomer
ggccaugcauguguucagauu

SEQ ID NO: 54 - RNA, 21 nt, Artificial Sequence
  Description of Artificial Sequence: Synthetic P15U16 sense oligonucleotide
  modified_base (1)..(1): Non-nucleotide monomer
  modified_base (20)..(20): Non-nucleotide monomer
ggccaugcauguguucagauu

SEQ ID NO: 55 - DNA, 21 bp, Artificial Sequence
  Description of Artificial Sequence: Synthetic siRNA P15 antisense oligonucleotide
  Description of Combined DNA/RNA Molecule: Synthetic siRNA P15 antisense oligonucleotide
ucugaacacaugcauggcctt

SEQ ID NO: 56 - RNA, 21 nt, Artificial Sequence
  Description of Artificial Sequence: Synthetic P15U6 antisense oligonucleotide
  modified_base (6)..(6): Non-nucleotide monomer
  modified_base (20)..(20): Non-nucleotide monomer
ucugaacacaugcauggccuu

SEQ ID NO: 57 - RNA, 21 nt, Artificial Sequence
  Description of Artificial Sequence: Synthetic P15U7 antisense oligonucleotide
  modified_base (7)..(7): Non-nucleotide monomer
  modified_base (20)..(20): Non-nucleotide monomer
ucugaacacaugcauggccuu

SEQ ID NO: 58 - RNA, 21 nt, Artificial Sequence
  Description of Artificial Sequence: Synthetic P15U14 antisense oligonucleotide
  modified_base (14)..(14): Non-nucleotide monomer
  modified_base (20)..(20): Non-nucleotide monomer
ucugaacacaugcauggccuu

SEQ ID NO: 59 - RNA, 21 nt, Artificial Sequence
  Description of Artificial Sequence: Synthetic P15U15 antisense oligonucleotide
  modified_base (15)..(15): Non-nucleotide monomer
  modified_base (20)..(20): Non-nucleotide monomer
ucugaacacaugcauggccuu

SEQ ID NO: 60 - RNA, 21 nt, Artificial Sequence
  Description of Artificial Sequence: Synthetic P15U16 antisense oligonucleotide
  modified_base (16)..(16): Non-nucleotide monomer
  modified_base (20)..(20): Non-nucleotide monomer
ucugaacacaugcauggccuu

SEQ ID NO: 61 - DNA, 21 bp, Artificial Sequence
  Description of Artificial Sequence: Synthetic siRNA P16 sense oligonucleotide
  Description of Combined DNA/RNA Molecule: Synthetic siRNA P16 sense oligonucleotide
gccaugcauguguucagaatt

SEQ ID NO: 62 - RNA, 21 nt, Artificial Sequence
  Description of Artificial Sequence: Synthetic P16U6 sense oligonucleotide
  modified_base (1)..(1): Non-nucleotide monomer
  modified_base (20)..(20): Non-nucleotide monomer
gccaugcauguguucagaauu

SEQ ID NO: 63 - RNA, 21 nt, Artificial Sequence
  Description of Artificial Sequence: Synthetic P16U7 sense oligonucleotide
  modified_base (1)..(1): Non-nucleotide monomer
  modified_base (20)..(20): Non-nucleotide monomer
gccaugcauguguucagaauu

SEQ ID NO: 64 - RNA, 21 nt, Artificial Sequence
  Description of Artificial Sequence: Synthetic P16U15 sense oligonucleotide
  modified_base (1)..(1): Non-nucleotide monomer
  modified_base (20)..(20): Non-nucleotide monomer
gccaugcauguguucagaauu

SEQ ID NO: 65 - RNA, 21 nt, Artificial Sequence
  Description of Artificial Sequence: Synthetic P16U16 sense oligonucleotide
  modified_base (1)..(1): Non-nucleotide monomer
  modified_base (20)..(20): Non-nucleotide monomer
gccaugcauguguucagaauu

SEQ ID NO: 66 - RNA, 21 nt, Artificial Sequence
  Description of Artificial Sequence: Synthetic P16U17 sense oligonucleotide
  modified_base (1)..(1): Non-nucleotide monomer
  modified_base (20)..(20): Non-nucleotide monomer
gccaugcauguguucagaauu

SEQ ID NO: 67 - DNA, 21 bp, Artificial Sequence
  Description of Artificial Sequence: Synthetic siRNA P16 antisense oligonucleotide
  Description of Combined DNA/RNA Molecule: Synthetic siRNA P16 antisense oligonucleotide
uucugaacacaugcauggctt

SEQ ID NO: 68 - RNA, 21 nt, Artificial Sequence
  Description of Artificial Sequence: Synthetic P16U6 antisense oligonucleotide
  modified_base (6)..(6): Non-nucleotide monomer
  modified_base (20)..(20): Non-nucleotide monomer
uucugaacacaugcauggcuu

SEQ ID NO: 69 - RNA, 21 nt, Artificial Sequence
  Description of Artificial Sequence: Synthetic P16U7 antisense oligonucleotide
  modified_base (7)..(7): Non-nucleotide monomer
  modified_base (20)..(20): Non-nucleotide monomer
uucugaacacaugcauggcuu

SEQ ID NO: 70 - RNA, 21 nt, Artificial Sequence
  Description of Artificial Sequence: Synthetic P16U15 antisense oligonucleotide
  modified_base (15)..(15): Non-nucleotide monomer
  modified_base (20)..(20): Non-nucleotide monomer
uucugaacacaugcauggcuu

SEQ ID NO: 71 - RNA, 21 nt, Artificial Sequence
  Description of Artificial Sequence: Synthetic P16U16 antisense oligonucleotide
  modified_base (16)..(16): Non-nucleotide monomer
  modified_base (20)..(20): Non-nucleotide monomer
uucugaacacaugcauggcuu

SEQ ID NO: 72 - RNA, 21 nt, Artificial Sequence
  Description of Artificial Sequence: Synthetic P16U17 antisense oligonucleotide
  modified_base (17)..(17): Non-nucleotide monomer
  modified_base (20)..(20): Non-nucleotide monomer
uucugaacacaugcauggcuu